European Patent Application EP 4 470 628 A2, published December 4, 2024. Title: FRAGRANCE RELEASE MECHANISM, METHOD AND USES THEREOF. Applicant: UNIVERSIDADE DO MINHO. Application EP P900.0 EP2, filed October 11, 2024. The sequence listing filed with the application follows.

SEQUENCE LISTING (22 sequences)

SEQ ID NO: 1 - protein, 157 aa, Sus scrofa domesticus
  REGION 1..157: note = Pig OBP (PDB ID 1DZK)
QEPQPEQDPFELSGKWITSYIGSSDLEKIGENAPFQVFMRSIEFDDKESKVYLNFFSKENGICEEFSLIGTKQEGNTYDVNYAGNNKFVVSYASETALIISNINVDEEGDKTIMTGLLGKGTDIEDQDLEKFKEVTRENGIPEENIVNIIERDDCPA

SEQ ID NO: 2 - protein, 170 aa, Homo sapiens
  REGION 1..170: note = Human OBPIIa (UniProt ID Q9NY56)
MKTLFLGVTLGLAAALSFTLEEEDITGTWYVKAMVVDKDFPEDRRPRKVSPVKVTALGGGNLEATFTFMREDRCIQKKILMRKTEEPGKFSAYGGRKLIYLQELPGTDDYVFYCKDQRRGGLRYMGKLVGRNPNTNLEALEEFKKLVQHKGLSEEDIFMPLQTGSCVLEH

SEQ ID NO: 3 - protein, 170 aa, Homo sapiens
  REGION 1..170: note = Human OBPIIb (UniProt ID Q9NPH6)
MKTLFLGVTLGLAAALSFTLEEEDITGTWYVKAMVVDKDFPEDRRPRKVSPVKVTALGGGKLEATFTFMREDRCIQKKILMRKTEEPGKYSAYGGRKLMYLQELPRRDHYIFYCKDQHHGGLLHMGKLVGRNSDTNREALEEFKKLVQRKGLSEEDIFTPLQTGSCVPEH

SEQ ID NO: 4 - protein, 163 aa, Mus musculus
  REGION 1..163: note = Mouse OBP (UniProt ID OBP1A)
MAKFLLLALTFGLAHAAMEGPWKTVAIAADRVDKIERGGELRIYCRSLTCEKECKEMKVTFYVNENGQCSLTTITGYLQEDGKTYKTQFQGNNRYKLVDESPENLTFYSENVDRADRKTKLLFILGHGPLTSEQKEKFAELAEEKGIPAGNIREVLITDYCPE

SEQ ID NO: 5 - protein, 176 aa, Mus musculus
  REGION 1..176: note = Mouse OBP2A (UniProt ID Q8K1H9)
MKSLLLTILLLGLVAVLKAQEAPPDDLVDYSGIWYAKAMVHNGTLPSHKIPSIVFPVRIIALEEGDLETTVVFWNNGHCREFKFVMKKTEEPGKYTAFHNTKVIHVEKTSVNEHYIFYCEGRHNGTSSFGMGKLMGRDSGENPEAMEEFKNFIKRMNLRLENMFVPEIGDKCVESD

SEQ ID NO: 6 - protein, 171 aa, Mus musculus
  REGION 1..171: note = Mouse OBP1B (UniProt ID A2AEP0)
MMVKFLLLALVFGLAHVHAHDHPELQGQWKTTAIMADNIDKIETSGPLELFVREITCDEGCQKMKVTFYVKQNGQCSLTTVTGYKQEDGKTFKNQYEGENNYKLLKATSENLVFYDENVDRASRKTKLLYILGKGEALTHEQKERLTELATQKGIPAGNLRELAHEDTCPE

SEQ ID NO: 7 - protein, 157 aa, Rattus rattus
  REGION 1..157: note = Rat OBP (PDB ID 3FIQ)
HHENLDISPSEVNGDWRTLYIVADNVEKVAEGGSLRAYFQHMECGDECQELKIIFNVKLDSECQTHTVVGQKHEDGRYTTDYSGRNYFHVLKKTDDIIFFHNVNVDESGKETNVILVAGKREDLNKAQKQELRKLAEEYNIPNENTQHLVPTDTCNQ

SEQ ID NO: 8 - protein, 173 aa, Rattus rattus
  REGION 1..173: note = Rat OBP (PDB ID 3ZQ3)
MRGSHHHHHHTDPEEASFERGNLDVDKLNGDWFSIVVASDKREKIEENGSMRVFVQHIDVLENSLGFTFRIKENGVCTEFSLVADKTAKDGEYFVEYDGENTFTILKTDYDNYVMFHLVNVNNGETFQLMELYGRTKDLSSDIKEKFAKLCVAHGITRDNIIDLTKTDRCLQA

SEQ ID NO: 9 - protein, 172 aa, Rattus rattus
  REGION 1..172: note = Rat OBP (UniProt ID P08937)
MVKFLLIVLALGVSCAHHENLDISPSEVNGDWRTLYIVADNVEKVAEGGSLRAYFQHMECGDECQELKIIFNVKLDSECQTHTVVGQKHEDGRYTTDYSGRNYFHVLKKTDDIIFFHNVNVDESGRRQCDLVAGKREDLNKAQKQELRKLAEEYNIPNENTQHLVPTDTCNQ

SEQ ID NO: 10 - protein, 159 aa, Bos gaurus
  REGION 1..159: note = Bovine OBP (PDB ID 1OBP)
AQEEEAEQNLSELSGPWRTVYIGSTNPEKIQENGPFRTYFRELVFDDEKGTVDFYFSVKRDGKWKNVHVKATKQDDGTYVADYEGQNVFKIVSLSRTHLVAHNINVDKHGQTTELTGLFVKLNVEDEDLEKFWKLTEDKGIDKKNVVNFLENEDHPHPE

SEQ ID NO: 11 - protein, 175 aa, Sus scrofa domesticus
  REGION 1..175: note = Boar OBP (PDB ID 1GM6)
HKEAGQDVVTSNFDASKIAGEWYSILLASDAKENIEENGSMRVFVEHIRVLDNSSLAFKFQRKVNGECTDFYAVCDKVGDGVYTVAYYGENKFRLLEVNYSDYVILHLVDVNGDKTFQLMEFYGRKPDVEPKLKDKFVEICQQYGIIKENIIDLTKIDRCFQLRGSGGVQESSAE

SEQ ID NO: 12 - protein, 168 aa, Ailuropoda melanoleuca
  REGION 1..168: note = Panda OBP (PDB ID 5NGH)
HEEGNDVRRNFDVSKISGYWYSVLLASDVREKTEENSSMRVFVNHIEVLSNSSLLFNMHIKVDGKCTEIALVSDKTEKDGEYSVEYDGYNVFRIVETDYTDYIIFHLVNFKEKDSFQMMELSAREPDTSEEVRKRFVEYCQKHGIVKENIFDLTEVDRCLQARGSEKA

SEQ ID NO: 13 - protein, 173 aa, Cricetulus griseus
  REGION 1..173: note = Chinese hamster OBP (Ensembl ID ENSCGRP00015014591.1)
MVKFLLLAFALSVSCAHHKIPEISPSEVDGKWRTLYIGADNTEKVIQGGPLRAYFRHMECSDECQTLTITFNTKEEGKCQTHTVVGRKDEDGQYKTGFSGNNDFHVVEKADGIIIFHNVNVDSSGKKTNVILVAGKGKSLSKEQKERLENIAKEFDISKENIQHLVPTDTCDQ

SEQ ID NO: 14 - protein, 173 aa, Sus scrofa domesticus
  REGION 1..173: note = Meishan pig OBP (Ensembl ID ENSSSCP00040041163.1)
MKSLLLSLVLGLVCAQEPQPEQDPFVLSGKWITSYIGSSDLEKIGENAPFQVFMRSIEFDDKESKVYLNFFSKENGICEEFSLIGTKQEGNTYDVNYAGNNKFVVSYASETALIISNINVDEEGDKTIMTGLLGKGTDIEDQDLEKFKEVTRENGIPEENIVNIIERDDCPAK

SEQ ID NO: 15 - protein, 175 aa, Equus caballus
  REGION 1..175: note = Horse OBP (Ensembl ID ENSECAP00000000103.2)
MQILLLSLVLGVVCAVQEPQSETDYSLFSGEWNTIYIGSSNIEKISENGPFRILLRRLDLDSAGDRIIYTFFLKVNGQCTKISSLAIKTEENTYVCHYAGKNKFEILHLSKTAIIIDIVNEDEGGLVTKMVALVGMLGDIQKEDIEKFKEVAKEKEIPEENIVNIINIDDCPTSE

SEQ ID NO: 16 - protein, 170 aa, Cavia porcellus
  REGION 1..170: note = Guinea pig OBP ((Ensembl ID ENSCPOP00000016393.2)
MQILLLALTIGLAYAHQTLDPSEINGQWHTISIAADNVEKIGEGGPLRGYFHNLHCYDGCKNIGLTFYVKLDGNCQRFDVLGAKQEDSDVYVAQYSGTNHFEVIGKKEDAIAFYNHNTDETGKETKMIVVVARRDSLTEEEQQKLQEVAGEKGIPKDNIRYFRERDTCAQ

SEQ ID NO: 17 - protein, 174 aa, Canis lupus
  REGION 1..174: note = Dog OBP ((Ensembl ID ENSCAFP00040020992.1)
MKILLLCLILVLACDAHLPLPNVLTQVSGPWKTLYVSSNNLDKIAENGPFRIYIRRINVDIPRLKILFSFFVKVDGECVEKSVEASIGQDNLINAHYAGGNYHQILDVTPNALIGYIVNVDDKGRITKLASLVGRGAHVNEEDIAKFKKLSREKGIPEENIIYLGDTDNCPNHE

SEQ ID NO: 18 - protein, 173 aa, Sus scrofa domesticus
  REGION 1..173: note = Tibetan pig OBP (Ensembl ID ENSSSCP00015013912.1)
MKSLLLSLVLGLVCAQEPQPEQDPFELSGKWITSYIGSSDLEKIGENAPFQVFMRSIEFDDKESKVYLNFFSKENGICEEFSLTGTKQEGNTYDVNYAGNNKFVVSYASETALIIANINVDEEGDKTIMTGLLGKGTDIEDQDLEKFKEVTRENGIPEENIVNIIERDDCPAK

SEQ ID NO: 19 - protein, 314 aa, Sus scrofa domesticus
  REGION 1..314: note = Cat felis OBP (Ensembl ID ENSFCAP00000053707.1)
RSCVIHLQCLPTGCLFSALHNGLPDGRLPLPDGRLPLPDGRLPLPDSRLPLPDGRLPLPDGRLPLPDGRLPLPDGRLPLPDGRLPLPDGRLPLPDGRLPLPDGRLPLPEGRLPLPDSHPPLQDNLTQLSGEWNTLLVAATNVDKISNGPFHGYICKVDVDVTNGTVVFNFSVMMNGRCTEKSAVGTIGRDKFINIGSMNQNLFNLFSVTSNTIAINVNTRRNTTKAFALLDTNGNIFNIGYDSLGSLIIHTANVDTAGQTTQVFALLGKRLHPDDNDFAKFRELMRENNIPEENLIDMSKTEKCPKKEKGTNPS

SEQ ID NO: 20 - protein, 175 aa, Pan troglodytes
  REGION 1..175: note = Chimpanzee OBP (Ensembl ID ENSPTRP00000048681.3)
MALLLLSLGLSLITAQEFDPRNVMQRNYNMARVSGVWYSIFMADDLNRIKENGDLRVFVQNIEHLKNGSLKFDFEYMVQGECVAVVVVCEKTEKNGEYSINYEGQNTVAVSETDYRLFITFHLQNFRNGTETHTLALYETCKKYGLGSQNIINLTNKDPCYSKHYRSPPRPPMRE

SEQ ID NO: 21 - protein, 210 aa, synthetic construct
  REGION 1..210: note = OBP::GQ20::KP (recombinant protein)
QEPQPEQDPFELSGKWITSYIGSSDLEKIGENAPFQVFMRSIEFDDKESKVYLNFFSKENGICEEFSLIGTKQEGNTYDVNYAGNNKFVVSYASETALIISNINVDEEGDKTIMTGLLGKGTDIEDQDLEKFKEVTRENGIPEENIVNIIERDDCPAGQGQGQGQGQGQGQGQGQGQGQGQGQGQGQGQGQGQGQGQGGVCGPSPPCITT

SEQ ID NO: 22 - protein, 349 aa, synthetic construct
  REGION 1..349: note = OBP::GQ20::CBM (recombinant protein)
QEPQPEQDPFELSGKWITSYIGSSDLEKIGENAPFQVFMRSIEFDDKESKVYLNFFSKENGICEEFSLIGTKQEGNTYDVNYAGNNKFVVSYASETALIISNINVDEEGDKTIMTGLLGKGTDIEDQDLEKFKEVTRENGIPEENIVNIIERDDCPAGQGQGQGQGQGQGQGQGQGQGQGQGQGQGQGQGQGQGQGQASPIGEGTFDDGPEGWVAYGTDGPLDTSTGALCVAVPAGSAQYGVGVVLNGVAIEEGTTYTLRYTATASTDVTVRALVGQNGAPYGTVLDTSPALTSEPRQVTETFTASATYPATPAADDPEGQIAFQLGGFSADAWTLCLDDVALDSEVEL